European Patent Application EP 4 756 010 A1, published June 10, 2026. Title: 菌株、培养物及其应用. Applicant: 慕恩（广州）生物科技有限公司. The sequence listing filed with the application follows.

SEQUENCE LISTING (7 sequences)

SEQ ID NO: 1 - DNA, 1540 bp, synthetic construct
  source 1..1540: mol_type = other DNA
aactttattagagagtttgatcctggctcaggatgaacgctggcggcgtgcttaacacatgcaagtcgaacgaagcgcttgagaagatttcttcggaatgaaacttaagtgactgagtggcggacgggtgagtaacgcgtgggtaacctgcctcatacagggggataacagtcagaaatgactgctaataccgcataagcgcacagtaccgcatggtacggtgtgaaaaactccggtggtatgggatggacccgcgtctgattagctagttggtggggtaacggcctaccaaggcgacgatcagtagccggcctgagagggcgaccggccacattgggactgagacacggcccaaactcctacgggaggcagcagtggggaatattgcacaatgggggaaaccctgatgcagcgacgccgcgtgagcgaagaagtatttcggtatgtaaagctctatcagcagggaagaaaatgacggtacctgactaagaagccccggctaactacgtgccagcagccgcggtaatacgtagggggcaagcgttatccggatttactgggtgtaaagggagcgtagacggactggcaagtctgatgtgaaaacccggggctcaaccccgggactgcattggaaactgtcagtctagagtgtcggaggggtaagtggaattcctagtgtagcggtgaaatgcgtagatattaggaggaacaccagtggcgaaggcggcttactggacgataactgacgttgaggctcgaaagcgtggggagcaaacaggattagataccctggtagtccacgccgtaaacgatgaatactaggtgtcgggaagcaaagcttttcggtgccgcagcaaacgcaataagtattccacctggggagtacgttcgcaagaatgaaactcaaaggaattgacggggacccgcacaagcggtggagcatgtggtttaattcgaagcaacgcgaagaaccttaccaagtcttgacatcgatctgcccggactgtaacgagtcctttcccttcggggacagagaagacaggtggtgcatggttgtcgtcagctcgtgtcgtgagatgttgggttaagtcccgcaacgagcgcaacccttatccttagtagccagcaggtaaagctgggcactctggggagactgccagggataacctggaggaaggtggggatgacgtcaaatcatcatgccccttatgatttgggctacacacgtgctacaatggcgtaaacaaagggaagcagccccgcgagggtgagcaaatctcaaaaataacgtcccagttcggattgtagtctgcaactcgactacatgaagctggaatcgctagtaatcgcaggtcagcatactgcggtgaatacgttcccgggtcttgtacacaccgcccgtcacaccatgggagtcggatatgcccgaagccagtgacccaaccttagggagggagctgtcgaaggtggagccgataactggggtgaagtcgtaacaaggtagccgtatcggaaggtgcggctggatcacctcctttct

SEQ ID NO: 2 - DNA, 21 bp, synthetic construct
  source 1..21: mol_type = other DNA
ctctgttcagctattggacgc

SEQ ID NO: 3 - DNA, 23 bp, synthetic construct
  source 1..23: mol_type = other DNA
cggaatttctgggattcagcttc

SEQ ID NO: 4 - DNA, 22 bp, synthetic construct
  source 1..22: mol_type = other DNA
cattggcttgcgagacgtagac

SEQ ID NO: 5 - DNA, 22 bp, synthetic construct
  source 1..22: mol_type = other DNA
gctgaaggtctcttccatcacc

SEQ ID NO: 6 - DNA, 21 bp, synthetic construct
  source 1..21: mol_type = other DNA
gtgttcctacccccaatgtgt

SEQ ID NO: 7 - DNA, 24 bp, synthetic construct
  source 1..24: mol_type = other DNA
attgtcataccaggaaatgagctt